European Patent Specification EP 3 523 440 B1, published January 29, 2025. Title: EARLY POST-TRANSFECTION ISOLATION OF CELLS (EPIC) FOR BIOLOGICS PRODUCTION. Applicant: Genzyme Corporation. The sequence listing filed with the application follows.

SEQUENCE LISTING (8 sequences)

SEQ ID NO: 1 - DNA, 10 bp, Artificial sequence
  Synthetic oligonucleotide
gccrccatgg

SEQ ID NO: 2 - protein, 61 aa, Homo sapiens
LERFLFLLLTISLLVLVQIQTGLSGQNDTSQTSSPSASSNISGGIFLFFVANAIIHLFCFS

SEQ ID NO: 3 - protein, 128 aa, Homo sapiens
LGIQGGSVLFGLLLVLAVFCHSGHSLQCYNCPNPTADCKTAVNCSSDFDACLITKAGLQVYNNCWKFEHCNFNDVTTRLRENELTYYCCKKDLCNFNEQLENGGTSLSEKTVLLLVTPFLAAAWSLHP

SEQ ID NO: 4 - protein, 74 aa, Mus musculus
LKSFLLFLTIILLVVIQIQTGSLGQATTAASGTNKNSTSTKKTPLKSGASSIIDAGACSFLFFANTLICLFYLS

SEQ ID NO: 5 - protein, 74 aa, Homo sapiens; identical to SEQ ID NO: 4

SEQ ID NO: 6 - DNA, 387 bp, Homo sapiens
ttgggaatccaaggagggtctgtcctgttcgggctgctgctcgtcctcgctgtcttctgccattccggtcatagcctgcagtgctacaactgtcctaacccaactgctgactgcaaaacagccgtcaattgttcatctgattttgacgcgtgtctcattaccaaagctgggttacaagtgtataacaactgttggaagtttgagcattgcaatttcaacgacgtcacaacccgcttgagggaaaacgagctaacgtactactgctgcaagaaggacctgtgtaactttaacgaacagcttgaaaacggagggacatccttatcagagaaaacagttcttctgctggtgactccatttctggcagctgcttggagccttcatccctaa

SEQ ID NO: 7 - DNA, 233 bp, Mus musculus
ttgaagagcttcctcctcttcctcactatcattcttctcgtagtcattcagatacaaacaggatccttaggacaagccactacggccgcttcaggtactaacaaaaacagcacctccaccaaaaaaacccccttaaagagcggggcctcatccatcatcgacgcgggcgcttgcagtttcctcttcttcgccaatacccttatttgcctcttctacctcagctaactgagtaa

SEQ ID NO: 8 - DNA, 8123 bp, Artificial sequence
  Synthetic polynucleotide
ggatccgctgtggaatgtgtgtcagttagggtgtggaaagtccccaggctccccagcaggcagaagtatgcaaagcatgcatctcaattagtcagcaaccaggtgtggaaagtccccaggctccccagcaggcagaagtatgcaaagcatgcatctcaattagtcagcaaccatagtcccgcccctaactccgcccatcccgcccctaactccgcccagttccgcccattctccgccccatggctgactaattttttttatttatgcagaggccgaggccgcctcggcctctgagctattccagaagtagtgaggaggcttttttggaggcctaggcttttgcaaaaagcttggggggggggacagctcagggctgcgatttcgcgccaaacttgacggcaatcctagcgtgaaggctggtaggattttatccccgctgccatcatggttcgaccattgaactgcatcgtcgccgtgtcccaaaatatggggattggcaagaacggagacctaccctggcctccgctcaggaacgagttcaagtacttccaaagaatgaccacaacctcttcagtggaaggtaaacagaatctggtgattatgggtaggaaaacctggttctccattcctgagaagaatcgacctttaaaggacagaattaatatagttctcagtagagaactcaaagaaccaccacgaggagctcattttcttgccaaaagtttggatgatgccttaagacttattgaacaaccggaattggcaagtaaagtagacatggtttggatagtcggaggcagttctgtttaccaggaagccatgaatcaaccaggccacctcagactctttgtgacaaggatcatgcaggaatttgaaagtgacacgtttttcccagaaattgatttggggaaatataaacttctcccagaatacccaggcgtcctctctgaggtccaggaggaaaaaggcatcaagtataagtttgaagtctacgagaagaaagactaacaggaagatgctttcaagttctctgctcccctcctaaagctatgcatttttataagaccatgggacttttgctggctttagatctttgtgaaggaaccttacttctgtggtgtgacataattggacaaactacctacagagatttaaagctctaaggtaaatataaaatttttaagtgtataatgtgttaaactactgattctaattgtttgtgtattttagattccaacctatggaactgatgaatgggagcagtggtggaatgcctttaatgaggaaaacctgttttgctcagaagaaatgccatctagtgatgatgaggctactgctgactctcaacattctactcctccaaaaaagaagagaaaggtagaagaccccaaggactttccttcagaattgctaagttttttgagtcatgctgtgtttagtaatagaactcttgcttgctttgctatttacaccacaaaggaaaaagctgcactgctatacaagaaaattatggaaaaatattctgtaacctttataagtaggcataacagttataatcataacatactgttttttcttactccacacaggcatagagtgtctgctattaataactatgctcaaaaattgtgtacctttagctttttaatttgtaaaggggttaataaggaatatttgatgtatagtgccttgactagagatcataatcagccataccacatttgtagaggttttacttgctttaaaaaacctcccacacctccccctgaacctgaaacataaaatgaatgcaattgttgttgttaacttgtttattgcagcttataatggttacaaataaagcaatagcatcacaaatttcacaaataaagcatttttttcactgcattctagttgtggtttgtccaaactcatcaatgtatcttatcatgtctggatcctctacgccggacgcatcgtggccggcatcaccggcgccacaggtgcggttgctggcgcctatatcgccgacatcaccgatggggaagatcgggctcgccacttcgggctcatgagcgcttgtttcggcgtgggtatggtggcaggccgtggccgggggactgttgggcgccatctccttgcatgcaccattccttgcggcggcggtgctcaacggcctcaacctactactgggctgcttcctaatgcaggagtcgcataagggagagcgtcgaccgatgcccttgagagccttcaacccagtcagctccttccggtgggcgcggggcatgactatcgtcgccgcacttatgactgtcttctttatcatgcaactcgtaggacaggtgccggcagcgctctgggtcattttcggcgaggaccgctttcgctggagcgcgacgatgatcggcctgtcgcttgcggtattcggaatcttgcacgccctcgctcaagccttcgtcactggtcccgccaccaaacgtttcggcgagaagcaggccattatcgccggcatggcggccgacgcgctgggctacgtcttgctggcgttcgcgacgcgaggctggatggccttccccattatgattcttctcgcttccggcggcatcgggatgcccgcgttgcaggccatgctgtccaggcaggtagatgacgaccatcagggacagcttcaaggccagcaaaaggccaggaaccgtaaaaaggccgcgttgctggcgtttttccataggctccgcccccctgacgagcatcacaaaaatcgacgctcaagtcagaggtggcgaaacccgacaggactataaagataccaggcgtttccccctggaagctccctcgtgcgctctcctgttccgaccctgccgcttaccggatacctgtccgcctttctcccttcgggaagcgtggcgctttctcatagctcacgctgtaggtatctcagttcggtgtaggtcgttcgctccaagctgggctgtgtgcacgaaccccccgttcagcccgaccgctgcgccttatccggtaactatcgtcttgagtccaacccggtaagacacgacttatcgccactggcagcagccactggtaacaggattagcagagcgaggtatgtaggcggtgctacagagttcttgaagtggtggcctaactacggctacactagaaggacagtatttggtatctgcgctctgctgaagccagttaccttcggaaaaagagttggtagctcttgatccggcaaacaaaccaccgctggtagcggtggtttttttgtttgcaagcagcagattacgcgcagaaaaaaaggatctcaagaagatcctttgatcttttctacggggtctgacgctcagtggaacgaaaactcacgttaagggattttggtcatgagattatcaaaaaggatcttcacctagatccttttaaattaaaaatgaagttttaaatcaatctaaagtatatatgagtaaacttggtctgacagttaccaatgcttaatcagtgaggcacctatctcagcgatctgtctatttcgttcatccatagttgcctgactccccgtcgtgtagataactacgatacgggagggcttaccatctggccccagtgctgcaatgataccgcgagacccacgctcaccggctccagatttatcagcaataaaccagccagccggaagggccgagcgcagaagtggtcctgcaactttatccgcctccatccagtctattaattgttgccgggaagctagagtaagtagttcgccagttaatagtttgcgcaacgttgttgccattgctgcaggcatcgtggtgtcacgctcgtcgtttggtatggcttcattcagctccggttcccaacgatcaaggcgagttacatgatcccccatgttgtgcaaaaaagcggttagctccttcggtcctccgatcgttgtcagaagtaagttggccgcagtgttatcactcatggttatggcagcactgcataattctcttactgtcatgccatccgtaagatgcttttctgtgactggtgagtactcaaccaagtcattctgagaatagtgtatgcggcgaccgagttgctcttgcccggcgtcaacacgggataataccgcgccacatagcagaactttaaaagtgctcatcattggaaaacgttcttcggggcgaaaactctcaaggatcttaccgctgttgagatccagttcgatgtaacccactcgtgcacccaactgatcttcagcatcttttactttcaccagcgtttctgggtgagcaaaaacaggaaggcaaaatgccgcaaaaaagggaataagggcgacacggaaatgttgaatactcatactcttcctttttcaatattattgaagcatttatcagggttattgtctcatgagcggatacatatttgaatgtatttagaaaaataaacaaataggggttccgcgcacatttccccgaaaagtgccacctgacgtctaagaaaccattattatcatgacattaacctataaaaataggcgtatcacgaggccctttcgtcttcaagaattggggaccaagacagaaccataagccagtgggatagatcagaaatgttccagaggtgggatggggccagagtgcctgccccttgaaccgtcccagggaccagaggtgacaaagtggcaacacaggtcctgcctgggaatctggtctgctcctacttagtaaagctgcctggtgtcacacaagaggcccccacttattcctgcacccctggtggtaggtggcgtcttctcccctgcagccaccaggctcccctgagaacactgccggcagtcctcattgacaggcagtattcgctctgccccacccccacctgtgaattgcagggctggcaggtcctcaggcagctggcaaaccgcctgaacaactgagagatacagggccagggccagggcagtcccgtcccccggaggcagggaggggacgtgctgggaaagttctctctctcaggcccaggttggtgactgcagaaggcttctgtcaaatctcttttgtgggaaccacagagtagccctgaacgtgggggtgtgcttccagtatactctggggtcaccctttccatactggaggcctctgcaacttcaaaatgctctgctaccaacctagcacaaggaagttggtccagcctccccacgcagggccactgctgcagtccatatatggactaagccttccttggtttcaacacctacactcactgagcccctactatgtgtatgcagagccgagacaggccctgagcatctcatctgaagcacccttcttgcctaaattcagttttctgtcactttctcccaggaggtgtgtgtccctctaagctaagccaggggtccctcacccctgccccactcccatccctagtgtaggtatcagctgaagagcttcctgagcagaacactcttgggtgctgacattttgataaataggcccatgtttaggagagcaggggtccgggggcgggagatcttctctggtggattgagggctccaagaactactctttgagcacgctgcccctcccagagtccccacagcctccagatggactagaacacagttcggctgtggctgcacataactaacagaggatagatggtgggtcccagcccaacagtgcctggcaatcacccagagccaccagctaacggccttggcttagttttttgcctgggtgtgatcaggcagccctccaaaactgcccggactccatgacaagttttgcttgttctatagagcacagttcctttctaggtctggggcaagggacatcgggagacatcttcctgcaacagctccagtcactggaccaccaggctcgccctgtctttggtgtgtggccctgagtctcctaagtggcccaaacctgtgaagacccctccaaccacagttttgcttctaaattgtaccccaacacacctagcaaattgaaaccccaccagaagtcccccagatctggctttccggctattgctggcaagggggagtgactcccggcccattcaatccaggccccgcgtgttcctcaaacaagaagccacgtaaacataaaccgagcctccatgctgacccttgcccatcgaggtactcaatgttcacgtgatatccacacccagagggtcctggggtgggtgcatgagccccagaatgcaggcttgataaccgagaccctgaatcgggcagtgtccacaagggcggaggccagtcatgcatgttcgggcctatggggccagcacccaacgccaaaactctccatcctcttcctcaatctcgctttctctctctctctctttttttttttttattttttttttttgcaaaaggaggggagagggggtaaaaaaatgctgcactgtgcggctaggccggtgagtgagcggcgcggagccaatcagcgctcgccgttccgaaagttgccttttatggctcgagtggccgctgtggcgtcctataaaacccggcggcgcaacgcgcagccactgtcgagtccgcgtccacccgcgagcacaggcctttcgcagctctttcttcgccgctccacacccgccaccaggtaagcagggacaacaggcccagccggccacagccctcccgtgggcagtgaccgcgctgcagggtcgcgggggacactcggcgcggacaccggggaaggctggagggtggtgccgggccgcggagcggacactttcagatccaactttcagtccagggtgtagaccctttacagccgcattgccacggtgtagacaccggtggacccgctctggctcagagcacgcggcttgggggaacccattagggtcgcagtgtgggcgctatgagagccgatgcagctttcgggtgttgaaccgtatctgcccaccttggggggaggacacaaggtcgggagccaaacgccacgatcatgccttggtggcccatgggtctttgtctaaaccggtttgcccatttggcttgccgggcgggcgggcgcggcgggcccggctcggccgggtgggggctgggttgccactgcgcttgcgcgctctatggctgggtattggggcgcgtgcacgctggggagggagcccttcctcttccccctctcccaagttaaacttgcgcgtgcgtattgagacttggagcgcggccaccggggttgggcgagggcggggccgttgtccggaaggggcggggtcgcagcggcttcggggcgcctgctcgcgcttcctgctgggtgtggtcgcctcccgcgcgcgcactagccgcccgccggcggggcgaaggcggggcttgcgcccgtttggggagggggcggaggcctggcttcctgccgtggggccgcctccggaccagcgtttgcctcttatggtaataacgcggccggcctgggcttcctttgtcccctgagtttgggcgcgcgccccctggcggcccgaggccgcggcttgccggaagtgggcagggcggcagcggctgcgcctagtggcccgctagtgaccgcgaccctcttttgtgccctgatatagttcgccggatcctaccgcggtagcggccgcgccaccttggagcgcttcctcttcctcctactcaccatcagcctcctcgttttggtacaaatacaaaccggactctccggacaaaacgacaccagccaaaccagcagcccctcagcatccagcaacataagcggaggcattttccttttcttcgtcgccaacgccataatccacctcttctgcttcagttgaaggccggccaatacgtaggcgcgccattgagtgagtgatttggcgcgccaagatatcacacccgggattaattaaaggtacctacgcgtagaattccacgtagtggtttaaactctagatactcgagggatctggatcataatcagccataccacatttgtagaggttttacttgctttaaaaaacctcccacacctccccctgaacctgaaacataaaatgaatgcaattgttgttgttaacttgtttattgcagcttataatggttacaaataaagcaatagcatcacaaatttcacaaataaagcatttttttcactgcattctagttgtggtttgtccaaactcatcaatgtatcttatcatgtct